European Patent Specification EP 3 766 989 B1, published January 1, 2025. Title: A method for screening compounds that control the function of RNA. Applicant: Veritas In Silico Inc. The sequence listing filed with the application follows.

SEQUENCE LISTING (19 sequences)

SEQ ID NO: 1 - RNA, 35 nt, Artificial Sequence
  potentially stem-loop forming sequence
gguggcggcggcggcaugggugccccgacguugcc

SEQ ID NO: 2 - RNA, 64 nt, Artificial Sequence
  potentially stem-loop forming sequence
gcagcccuuucucaaggaccaccgcaucucuacauucaagaacuggcccuucuuggagggcugc

SEQ ID NO: 3 - RNA, 52 nt, Artificial Sequence
  potentially stem-loop forming sequence
ggccgaggcuggcuucauccacugccccacugagaacgagccagacuuggcc

SEQ ID NO: 4 - RNA, 61 nt, Artificial Sequence
  potentially stem-loop forming sequence
uuucugucaagaagcaguuugaagaauuaacccuuggugaauuuuugaaacuggacagaga

SEQ ID NO: 5 - RNA, 28 nt, Artificial Sequence
  potentially stem-loop forming sequence
ggggcucauuuuugcuguuuugauuccc

SEQ ID NO: 6 - RNA, 72 nt, Artificial Sequence
  potentially stem-loop forming sequence
gugggggacuggcugggcugcugcaggccgugugucugucagcccaaccuucacaucugucacguucuccac

SEQ ID NO: 7 - RNA, 73 nt, Artificial Sequence
  potentially stem-loop forming sequence
gcagcucccgcagggcugaagucuggcguaagaugauggauuugauucgcccuccucccugucauagagcugc

SEQ ID NO: 8 - RNA, 20 nt, Artificial Sequence
  potentially stem-loop forming sequence
uuucccucuaaacugggaga

SEQ ID NO: 9 - RNA, 18 nt, Artificial Sequence
  potentially stem-loop forming sequence
ggccuuuccuuaaaggcc

SEQ ID NO: 10 - RNA, 35 nt, Artificial Sequence; identical to SEQ ID NO: 1
  potentially stem-loop forming sequence

SEQ ID NO: 11 - RNA, 48 nt, Artificial Sequence
  potentially stem-loop forming sequence
ggcagagguggcggcggcggcaugggugccccgacguugcccccugcc

SEQ ID NO: 12 - RNA, 35 nt, Artificial Sequence; identical to SEQ ID NO: 1
  potentially stem-loop forming sequence

SEQ ID NO: 13 - RNA, 41 nt, Artificial Sequence
  potentially stem-loop forming sequence
agagguggcggcggcggcaugggugccccgacguugccccc

SEQ ID NO: 14 - RNA, 19 nt, Artificial Sequence
  probe sequence
agagguggcggcggcggca

SEQ ID NO: 15 - RNA, 18 nt, Artificial Sequence
  probe sequence
ugccccgacguugccccc

SEQ ID NO: 16 - RNA, 20 nt, Artificial Sequence
  probe sequence
ggaugcuuacucagcgaucc

SEQ ID NO: 17 - RNA, 38 nt, Artificial Sequence
  probe sequence
ggaucccgacuggcgagagccagguaacgaauggaucc

SEQ ID NO: 18 - RNA, 35 nt, Artificial Sequence
  probe sequence
ggcguguaggauaugcuucggcagaaggacacgcc

SEQ ID NO: 19 - RNA, 21 nt, Artificial Sequence
  probe sequence
gggucucucuucggggaaccc